European Patent Application EP 4 559 927 A1, published May 28, 2025. Title: carrier peptide fragment and use thereof. Applicant: TOAGOSEI CO., LTD. The sequence listing filed with the application follows.

SEQUENCE LISTING (11 sequences)

SEQ ID NO: 1 - protein, 13 aa, synthetic construct
KKRTLRKSNRKKR

SEQ ID NO: 2 - protein, 13 aa, synthetic construct
KKRTLRKDERKKR

SEQ ID NO: 3 - protein, 13 aa, synthetic construct
KKRTLRKEDRKKR

SEQ ID NO: 4 - protein, 15 aa, synthetic construct
KKRTLRKEDEDRKKR

SEQ ID NO: 5 - protein, 15 aa, synthetic construct
KKRTLRKEEDDRKKR

SEQ ID NO: 6 - protein, 15 aa, synthetic construct
KKRTLRKDDEERKKR

SEQ ID NO: 7 - protein, 15 aa, synthetic construct
KKRTLRKDEDERKKR

SEQ ID NO: 8 - protein, 17 aa, synthetic construct
KKRTLRKEDEDEDRKKR

SEQ ID NO: 9 - protein, 13 aa, synthetic construct
KKRTLRKDDRKKR

SEQ ID NO: 10 - protein, 13 aa, synthetic construct
KKRTLRKEERKKR

SEQ ID NO: 11 - protein, 14 aa, synthetic construct
VVRSLVKVVRSLVK